European Patent Application EP 4 592 316 A1, published July 30, 2025. Title: 分离的抗原结合蛋白及其应用. Applicant: 广州凌腾生物医药有限公司. The sequence listing filed with the application follows.

SEQUENCE LISTING (40 sequences)

SEQ ID NO: 1 - protein, 5 aa, synthetic construct
NYWMT

SEQ ID NO: 2 - protein, 5 aa, synthetic construct
NYWMS

SEQ ID NO: 3 - protein, 17 aa, synthetic construct
SITKTGGSTYYPDSVKG

SEQ ID NO: 4 - protein, 17 aa, synthetic construct
AITKTGGSTYYADSVKG

SEQ ID NO: 5 - protein, 17 aa, synthetic construct
AITKTGGSTYYPDSVKG

SEQ ID NO: 6 - protein, 10 aa, synthetic construct
EYYYDPYIDY

SEQ ID NO: 7 - protein, 13 aa, synthetic construct
KRSTGNIGSNYVN

SEQ ID NO: 8 - protein, 13 aa, synthetic construct
TGTTGNIGSNYVS

SEQ ID NO: 9 - protein, 13 aa, synthetic construct
KRTTGNIGSNYVN

SEQ ID NO: 10 - protein, 13 aa, synthetic construct
TRTTGNIGSNYVN

SEQ ID NO: 11 - protein, 7 aa, synthetic construct
RDDKRPD

SEQ ID NO: 12 - protein, 7 aa, synthetic construct
RDDKRPS

SEQ ID NO: 13 - protein, 9 aa, synthetic construct
QSYSSGINI

SEQ ID NO: 14 - protein, 119 aa, synthetic construct
EVQLVESGGGLVQPGRSLKLSCVASGFTFNNYWMTWIRQAPGKGLEWVASITKTGGSTYYPDSVKGRFTISRDNAKSTLYLQMNSLRSEDTATYYCTREYYYDPYIDYWGQGVMVTVSS

SEQ ID NO: 15 - protein, 119 aa, synthetic construct
EVQLVESGGGLVQPGGSLRLSCAASGFTFNNYWMSWVRQAPGKGLEWVSAITKTGGSTYYADSVKGRFTISRDNSKNTLYLQMNSLRAEDTAVYYCTREYYYDPYIDYWGQGTLVTVSS

SEQ ID NO: 16 - protein, 119 aa, synthetic construct
EVQLVESGGGLVQPGRSLRLSCAASGFTFNNYWMSWVRQAPGKGLEWVSAITKTGGSTYYPDSVKGRFTISRDNSKSTLYLQMNSLRAEDTATYYCTREYYYDPYIDYWGQGVLVTVSS

SEQ ID NO: 17 - protein, 119 aa, synthetic construct
EVQLVESGGGLVQPGRSLRLSCAASGFTFNNYWMSWVRQAPGKGLEWVASITKTGGSTYYPDSVKGRFTISRDNAKSTLYLQMNSLRSEDTATYYCTREYYYDPYIDYWGQGVLVTVSS

SEQ ID NO: 18 - protein, 119 aa, synthetic construct
EVQLVESGGGLVQPGGSLRLSCAASGFTFNNYWMTWIRQAPGKGLEWVASITKTGGSTYYPDSVKGRFTISRDNSKSTLYLQMNSLRAEDTAVYYCTREYYYDPYIDYWGQGTLVTVSS

SEQ ID NO: 19 - protein, 110 aa, synthetic construct
QFVLSQPNSVSTNLGSTVKLSCKRSTGNIGSNYVNWYQQHEGRSPTTMIYRDDKRPDGVPDRFSGSIDRSSNSALLTINNVQTEDEADYFCQSYSSGINIFGGGTKLTVL

SEQ ID NO: 20 - protein, 108 aa, synthetic construct
QSALTQPRSVSGSPGQSVTISCTGTTGNIGSNYVSWYQQHPGKAPKLMIYRDDKRPSGVPDRFSGSKSGNTASLTISGLQAEDEADYYCQSYSSGINIFGGGTKLTVL

SEQ ID NO: 21 - protein, 110 aa, synthetic construct
QFALTQPRSVSGNLGSSVKISCKRTTGNIGSNYVNWYQQHEGKAPTTMIYRDDKRPDGVPDRFSGSKDRSGNTALLTINNLQTEDEADYYCQSYSSGINIFGGGTKLTVL

SEQ ID NO: 22 - protein, 110 aa, synthetic construct
QFALTQPRSVSGSLGQSVTLSCTRTTGNIGSNYVNWYQQHEGKAPKTMIYRDDKRPSGVPDRFSGSIDRSSNTASLTISGVQAEDEADYYCQSYSSGINIFGGGTKLTVL

SEQ ID NO: 23 - protein, 110 aa, synthetic construct
QSALTQPRSVSGSPGQSVTISCTRTTGNIGSNYVNWYQQHPGKAPKTMIYRDDKRPSGVPDRFSGSIDSSSNTASLTISGLQAEDEADYYCQSYSSGINIFGGGTKLTVL

SEQ ID NO: 24 - protein, 109 aa, synthetic construct
ASTKGPSVFPLAPSSKSTSGGTAALGCLVKDYFPEPVTVSWNSGALTSGVHTFPAVLQSSGLYSLSSVVTVPSSSLGTQTYICNVNHKPSNTKVDKKVEPKSCHHHHHH

SEQ ID NO: 25 - protein, 106 aa, synthetic construct
GQPKAAPSVTLFPPSSEELQANKATLVCLISDFYPGAVKVAWKADGSPVNTGVETTTPSKQSNNKYAASSYLSLTPEQWKSHRSYSCQVTHEGSTVEKTVAPAECS

SEQ ID NO: 26 - protein, 228 aa, synthetic construct
EVQLVESGGGLVQPGRSLKLSCVASGFTFNNYWMTWIRQAPGKGLEWVASITKTGGSTYYPDSVKGRFTISRDNAKSTLYLQMNSLRSEDTATYYCTREYYYDPYIDYWGQGVMVTVSSASTKGPSVFPLAPSSKSTSGGTAALGCLVKDYFPEPVTVSWNSGALTSGVHTFPAVLQSSGLYSLSSVVTVPSSSLGTQTYICNVNHKPSNTKVDKKVEPKSCHHHHHH

SEQ ID NO: 27 - protein, 228 aa, synthetic construct
EVQLVESGGGLVQPGGSLRLSCAASGFTFNNYWMSWVRQAPGKGLEWVSAITKTGGSTYYADSVKGRFTISRDNSKNTLYLQMNSLRAEDTAVYYCTREYYYDPYIDYWGQGTLVTVSSASTKGPSVFPLAPSSKSTSGGTAALGCLVKDYFPEPVTVSWNSGALTSGVHTFPAVLQSSGLYSLSSVVTVPSSSLGTQTYICNVNHKPSNTKVDKKVEPKSCHHHHHH

SEQ ID NO: 28 - protein, 228 aa, synthetic construct
EVQLVESGGGLVQPGRSLRLSCAASGFTFNNYWMSWVRQAPGKGLEWVSAITKTGGSTYYPDSVKGRFTISRDNSKSTLYLQMNSLRAEDTATYYCTREYYYDPYIDYWGQGVLVTVSSASTKGPSVFPLAPSSKSTSGGTAALGCLVKDYFPEPVTVSWNSGALTSGVHTFPAVLQSSGLYSLSSVVTVPSSSLGTQTYICNVNHKPSNTKVDKKVEPKSCHHHHHH

SEQ ID NO: 29 - protein, 228 aa, synthetic construct
EVQLVESGGGLVQPGRSLRLSCAASGFTFNNYWMSWVRQAPGKGLEWVASITKTGGSTYYPDSVKGRFTISRDNAKSTLYLQMNSLRSEDTATYYCTREYYYDPYIDYWGQGVLVTVSSASTKGPSVFPLAPSSKSTSGGTAALGCLVKDYFPEPVTVSWNSGALTSGVHTFPAVLQSSGLYSLSSVVTVPSSSLGTQTYICNVNHKPSNTKVDKKVEPKSCHHHHHH

SEQ ID NO: 30 - protein, 228 aa, synthetic construct
EVQLVESGGGLVQPGGSLRLSCAASGFTFNNYWMTWIRQAPGKGLEWVASITKTGGSTYYPDSVKGRFTISRDNSKSTLYLQMNSLRAEDTAVYYCTREYYYDPYIDYWGQGTLVTVSSASTKGPSVFPLAPSSKSTSGGTAALGCLVKDYFPEPVTVSWNSGALTSGVHTFPAVLQSSGLYSLSSVVTVPSSSLGTQTYICNVNHKPSNTKVDKKVEPKSCHHHHHH

SEQ ID NO: 31 - protein, 216 aa, synthetic construct
QFVLSQPNSVSTNLGSTVKLSCKRSTGNIGSNYVNWYQQHEGRSPTTMIYRDDKRPDGVPDRFSGSIDRSSNSALLTINNVQTEDEADYFCQSYSSGINIFGGGTKLTVLGQPKAAPSVTLFPPSSEELQANKATLVCLISDFYPGAVKVAWKADGSPVNTGVETTTPSKQSNNKYAASSYLSLTPEQWKSHRSYSCQVTHEGSTVEKTVAPAECS

SEQ ID NO: 32 - protein, 214 aa, synthetic construct
QSALTQPRSVSGSPGQSVTISCTGTTGNIGSNYVSWYQQHPGKAPKLMIYRDDKRPSGVPDRFSGSKSGNTASLTISGLQAEDEADYYCQSYSSGINIFGGGTKLTVLGQPKAAPSVTLFPPSSEELQANKATLVCLISDFYPGAVKVAWKADGSPVNTGVETTTPSKQSNNKYAASSYLSLTPEQWKSHRSYSCQVTHEGSTVEKTVAPAECS

SEQ ID NO: 33 - protein, 216 aa, synthetic construct
QFALTQPRSVSGNLGSSVKISCKRTTGNIGSNYVNWYQQHEGKAPTTMIYRDDKRPDGVPDRFSGSKDRSGNTALLTINNLQTEDEADYYCQSYSSGINIFGGGTKLTVLGQPKAAPSVTLFPPSSEELQANKATLVCLISDFYPGAVKVAWKADGSPVNTGVETTTPSKQSNNKYAASSYLSLTPEQWKSHRSYSCQVTHEGSTVEKTVAPAECS

SEQ ID NO: 34 - protein, 216 aa, synthetic construct
QFALTQPRSVSGSLGQSVTLSCTRTTGNIGSNYVNWYQQHEGKAPKTMIYRDDKRPSGVPDRFSGSIDRSSNTASLTISGVQAEDEADYYCQSYSSGINIFGGGTKLTVLGQPKAAPSVTLFPPSSEELQANKATLVCLISDFYPGAVKVAWKADGSPVNTGVETTTPSKQSNNKYAASSYLSLTPEQWKSHRSYSCQVTHEGSTVEKTVAPAECS

SEQ ID NO: 35 - protein, 216 aa, synthetic construct
QSALTQPRSVSGSPGQSVTISCTRTTGNIGSNYVNWYQQHPGKAPKTMIYRDDKRPSGVPDRFSGSIDSSSNTASLTISGLQAEDEADYYCQSYSSGINIFGGGTKLTVLGQPKAAPSVTLFPPSSEELQANKATLVCLISDFYPGAVKVAWKADGSPVNTGVETTTPSKQSNNKYAASSYLSLTPEQWKSHRSYSCQVTHEGSTVEKTVAPAECS

SEQ ID NO: 36 - protein, 119 aa, synthetic construct
EVQLVESGGGLVQPGGSLRLSCAASGFTFNNYWMSWVRQAPGKGLEWVANITKTGGSTYYVDSVKGRFTISRDNAKNSLYLQMNSLRAEDTAVYYCTREYYYDPYIDYWGQGTMVTVSS

SEQ ID NO: 37 - protein, 119 aa, synthetic construct
EVQLVESGGGLVQPGGSLRLSCAASGFTFNNYWMTWIRQAPGKGLEWVASITKTGGSTYYPDSVKGRFTISRDNAKNSLYLQMNSLRAEDTAVYYCTREYYYDPYIDYWGQGTMVTVSS

SEQ ID NO: 38 - protein, 119 aa, synthetic construct
EVQLVESGGGLVQPGGSLRLSCAASGFTFNNYWMTWIRQAPGKGLEWVASITKTGGSTYYPDSVKGRFTISRDNAKNSLYLQMNSLRAEDTATYYCTREYYYDPYIDYWGQGVMVTVSS

SEQ ID NO: 39 - protein, 110 aa, synthetic construct
NFMLTQPHSVSESPGKTVTISCTRSTGNIGSNYVQWYQQRPGSSPTTVIYRDDQRPSGVPDRFSGSIDSSSNSASLTISGLKTEDEADYYCQSYSSGINIFGGGTKLTVL

SEQ ID NO: 40 - protein, 110 aa, synthetic construct
QFVLSQPHSVSESPGKTVTISCKRSTGNIGSNYVNWYQQRPGSSPTTMIYRDDKRPSGVPDRFSGSIDRSSNSASLTISGLKTEDEADYFCQSYSSGINIFGGGTKLTVL